European Patent Application EP 4 793 346 A1, published August 19, 2026. Title: 一种糖基转移酶UGT76G1、UGT91C1突变体及其催化合成莱鲍迪苷A、D、M的方法. Applicant: 东台市浩瑞生物科技有限公司. The sequence listing filed with the application follows.

SEQUENCE LISTING (32 sequences)

SEQ ID NO: 1 - protein, 459 aa, synthetic construct
MAENKTETTVRRRRRIILFPVPFQGHINPILQLANVLYSKGFSITIFHTNFNKPKTSNYPHFTFRFILDNDPQDERISNLPTHGPLAGMRIPIINEHGADELRRELELLMLASEEDEEVSCLITDALWYFAQSVADSLNLRRLVLMTSSLFNFHAHVSLPQFDELGYLDPDDKTRLEEQASGFPMLKVKDIKSAYSNWQILKEILGKMIKQTKASSGVIWNSFKELEESELETVIREIPAPSFLIPLPKHLTASSSSLLDHDRTVFQWLDQQPPSSVLYVSFGSTSEVDEKDFLEIARGLVDSKQSFLWVVRPGFVKGSTWVEPLPDGFLGERGRIVKWVPQQEVLAHGAIGAFWTHSGWNSTLESVCEGVPMIFSDFGLDQPLNARYMSDVLKVGVYLENGWERGEIANAIRRVMVDEEGEYIRQNARVLKQKADVSLMKGGSSYESLESLVSYISSL

SEQ ID NO: 2 - DNA, 1380 bp, synthetic construct
  source 1..1380: mol_type = other DNA
atggccgaaaacaagaccgaaaccaccgtccgtcgtcgccgtcgtatcattctgttccctgttccgttccagggccatatcaacccgatcttacagctggcgaacgtactgtacagcaaaggcttcagcattaccattttccacaccaacttcaacaagccgaaaacttccaattacccgcacttcacgttccgtttcattctggacaatgacccgcaggacgagcgcattagtaacctgccgacacacggtccgctcgctggtatgcgtatcccaattatcaatgaacatggtgcagatgaactgcgtcgtgaactggaactgctgatgttagccagcgaagaagacgaagaagtctcgtgcctcatcaccgatgccctgtggtatttcgctcagtctgtagccgacagcctcaacttgcgtcgtctggtactgatgaccagctccctgtttaacttccacgctcacgtttctttgccgcaattcgatgagctgggttacctcgaccctgacgataaaactcgcctggaagaacaggcatctggttttccgatgctgaaagtaaaagatatcaagtctgcgtactccaactggcagatccttaaggaaatcctgggtaaaatgatcaaacagactaaagcgtctagcggtgtgatatggaactcctttaaagaactggaagaatctgaactggaaactgtaatccgtgaaatcccagctccgtctttcctgattccgctgccgaagcatctgaccgcttcctcttcgtcgctgctggaccacgatcgaactgtgtttcagtggctggatcagcaaccgccgtcttcggttctgtacgtgtctttcggttccacgagcgaagtggacgaaaaagacttcttagaaatcgcccgtggtctggtcgactctaaacaatctttcctgtgggtggttcgtccgggcttcgtgaaaggttctacctgggtagaaccgttgccggacggttttctgggtgaacgtggtcgtattgtgaagtgggtgccgcagcaggaagttctggcacatggcgcgatcggcgcgttttggacccactctggttggaacagcaccctggaatctgtttgcgaaggtgtaccgatgatcttctctgacttcggtttggaccagccgctcaacgcgcgttacatgtcagacgtactgaaagttggtgtttacctggagaacggttgggaacgtggcgaaatcgctaacgcgatccgccgtgtaatggttgatgaggaaggtgagtacatccgtcagaatgcacgtgtcctgaaacagaaagctgacgtgagtctgatgaaaggtgggtcctcctacgaaagcctggagtccctggtatcttacatttcctctttgtaa

SEQ ID NO: 3 - protein, 459 aa, synthetic construct
MAENKTETTVRRRRRIILFPVPFQGHINPILQLANVLYSKGFSITIFHTNFNKPKTSNYPHFTFRFILDNDPQDERISNLPTHGPLAGMRIPIINEHGADELRRELELQMLACEEDEEVSCLITDALWYFAQSVADSLNLRRLVLMTSSLFNFHAHVSLPQFDELGYLDPDDKTRLEEQASGFPMLKVKDIKSAYSNWQILKEILGKMIKQTKASSGVIWNSFKELEESELETVIREIPAPSFLIPLPKHLTASSSSLLDHDRTVFQWLDQQPPSSVLYVSFGSTSEVDEKDFLEIARGLVDSKQSFLWVVRPGFVKGSTWVEPLPDGFLGERGRIVKWVPQQEVLAHGAIGAFWTHSGWNSTLESVCEGVPMIFSDFGLDQPLNARYMSDVLKVGVYLENGWERGEIANAIRRVMVDEEGEYFRQNARVLKQKADVSLMKGGSSYESLESLVSYISSL

SEQ ID NO: 4 - DNA, 1380 bp, synthetic construct
  source 1..1380: mol_type = other DNA
atggccgaaaataaaacggagaccaccgttcgccggcgccggagaataatattattcccggtaccatttcaaggccacattaacccaattcttcagctagccaatgtgttgtactctaaaggattcagtatcaccatctttcacaccaacttcaacaaacccaaaacatctaattaccctcacttcactttcagattcatcctcgacaacgacccacaagacgaacgcatttccaatctaccgactcatggtccgctcgctggtatgcggattccgattatcaacgaacacggagctgacgaattacgacgcgaactggaactgcagatgttagcttgcgaagaagatgaagaggtatcgtgtttaatcacggatgctctttggtacttcgcgcaatctgttgctgacagtcttaacctccgacggcttgttttgatgacaagcagcttgtttaattttcatgcacatgtttcacttcctcagtttgatgagcttggttacctcgatcctgatgacaaaacccgtttggaagaacaagcgagtgggtttcctatgctaaaagtgaaagacatcaagtctgcgtattcgaactggcaaatactcaaagagatattagggaagatgataaaacaaacaaaagcatcttcaggagtcatctggaactcatttaaggaactcgaagagtctgagctcgaaactgttatccgtgagatcccggctccaagtttcttgataccactccccaagcatttgacagcctcttccagcagcttactagaccacgatcgaaccgtttttcaatggttagaccaacaaccgccaagttcggtactgtatgttagttttggtagtactagtgaagtggatgagaaagatttcttggaaatagctcgtgggttggttgatagcaagcagtcgtttttatgggtggttcgacctgggtttgtcaagggttcgacgtgggtcgaaccgttgccagatgggttcttgggtgaaagaggacgtattgtgaaatgggttccacagcaagaagtgctagctcatggagcaataggcgcattctggactcatagcggatggaactctacgttggaaagcgtttgtgaaggtgttcctatgattttctcggattttgggctcgatcaaccgttgaatgctagatacatgagtgatgttttgaaggtaggggtgtatttggaaaatgggtgggaaagaggagagatagcaaatgcaataagaagagttatggtggatgaagaaggagaatacttcagacagaatgcaagagttttgaaacaaaaggcagatgtttctttgatgaagggtggttcgtcttacgaatcattagagtctctagtttcttacatttcatcgttgtaa

SEQ ID NO: 5 - protein, 808 aa, synthetic construct
MANAERMITRVHSQRERLNETLVSERNEVLALLSRVEAKGKGILQQNQIIAEFEALPEQTRKKLEGGPFFDLLKSTQEAIVLPPWVALAVRPRPGVWEYLRVNLHALVVEELQPAEFLHFKEELVDGVKNGNFTLELDFEPFNASIPRPTLHKYIGNGVDFLNRHLSAKLFHDKESLLPLLKFLRLHSHQGKNLMLSEKIQNLNTLQHTLRKAEEYLAELKSETLYEEFEAKFEEIGLERGWGDNAERVLDMIRLLLDLLEAPDPCTLETFLGRVPMVFNVVILSPHGYFAQDNVLGYPDTGGQVVYILDQVRALEIEMLQRIKQQGLNIKPRILILTRLLPDAVGTTCGERLERVYDSEYCDILRVPFRTEKGIVRKWISRFEVWPYLETYTEDAAVELSKELNGKPDLIIGNYSDGNLVASLLAHKLGVTQCTIAHALEKTKYPDSDIYWKKLDDKYHFSCQFTADIFAMNHTDFIITSTFQEIAGSKETVGQYESHTAFTLPGLYRVVHGIDVFDPKFNIVSPGADMSIYFPYTEEKRRLTKFHSEIEELLYSDVENKEHLCVLKDKKKPILFTMARLDRVKNLSGLVEWYGKNTRLRELANLVVVGGDRRKESKDNEEKAEMKKMYDLIEEYKLNGQFRWISSQMDRVRNGELYRYICDTKGAFVQPALYEAFGLTVVEAMTCGLPTFATCKGGPAEIIVHGKSGFHIDPYHGDQAADTLADFFTKCKEDPSHWDEISKGGLQRIEEKYTWQIYSQRLLTLTGVYGFWKHVSNLDRLEARRYLEMFYALKYRPLAQAVPLAQDD

SEQ ID NO: 6 - DNA, 2427 bp, synthetic construct
  source 1..2427: mol_type = other DNA
atggcaaacgctgaacgtatgataacgcgcgtccacagccaacgtgagcgtttgaacgaaacgcttgtttctgagagaaacgaagtccttgccttgctttccagggttgaagccaaaggtaaaggtattttacaacaaaaccagatcattgctgaattcgaagctttgcctgaacaaacccggaagaaacttgaaggtggtcctttctttgaccttctcaaatccactcaggaagcaattgtgttgccaccatgggttgctctagctgtgaggccaaggcctggtgtttgggaatacttacgagtcaatctccatgctcttgtcgttgaagaactccaacctgctgagtttcttcatttcaaggaagaactcgttgatggagttaagaatggtaatttcactcttgagcttgatttcgagccattcaatgcgtctatccctcgtccaacactccacaaatacattggaaatggtgttgacttccttaaccgtcatttatcggctaagctcttccatgacaaggagagtttgcttccattgcttaagttccttcgtcttcacagccaccagggcaagaacctgatgttgagcgagaagattcagaacctcaacactctgcaacacaccttgaggaaagcagaagagtatctagcagagcttaagtccgaaacactgtatgaagagtttgaggccaagtttgaggagattggtcttgagaggggatggggagacaatgcagagcgtgtccttgacatgatacgtcttcttttggaccttcttgaggcgcctgatccttgcactcttgagacttttcttggaagagtaccaatggtgttcaacgttgtgatcctctctccacatggttactttgctcaggacaatgttcttggttaccctgacactggtggacaggttgtttacattcttgatcaagttcgtgctctggagatagagatgcttcaacgtattaagcaacaaggactcaacattaaaccaaggattctcattctaactcgacttctacctgatgcggtaggaactacatgcggtgaacgtctcgagagagtttatgattctgagtactgtgatattcttcgtgtgcccttcagaacagagaagggtattgttcgcaaatggatctcaaggttcgaagtctggccatatctagagacttacaccgaggatgctgcggttgagctatcgaaagaattgaatggcaagcctgaccttatcattggtaactacagtgatggaaatcttgttgcttctttattggctcacaaacttggtgtcactcagtgtaccattgctcatgctcttgagaaaacaaagtacccggattctgatatctactggaagaagcttgacgacaagtaccatttctcatgccagttcactgcggatattttcgcaatgaaccacactgatttcatcatcactagtactttccaagaaattgctggaagcaaagaaactgttgggcagtatgaaagccacacagcctttactcttcccggattgtatcgagttgttcacgggattgatgtgtttgatcccaagttcaacattgtctctcctggtgctgatatgagcatctacttcccttacacagaggagaagcgtagattgactaagttccactctgagatcgaggagctcctctacagcgatgttgagaacaaagagcacttatgtgtgctcaaggacaagaagaagccgattctcttcacaatggctaggcttgatcgtgtcaagaacttgtcaggtcttgttgagtggtacgggaagaacacccgcttgcgtgagctagctaacttggttgttgttggaggagacaggaggaaagagtcaaaggacaatgaagagaaagcagagatgaagaaaatgtatgatctcattgaggaatacaagctaaacggtcagttcaggtggatctcctctcagatggaccgggtaaggaacggtgagctgtaccggtacatctgtgacaccaagggtgcttttgtccaacctgcattatatgaagcctttgggttaactgttgtggaggctatgacttgtggtttaccgactttcgccacttgcaaaggtggtccagctgagatcattgtgcacggtaaatcgggtttccacattgacccttaccatggtgatcaggctgctgatactcttgctgatttcttcaccaagtgtaaggaggatccatctcactgggatgagatctcaaaaggagggcttcagaggattgaggagaaatacacttggcaaatctattcacagaggctcttgacattgactggtgtgtatggattctggaagcatgtctcgaaccttgaccgtcttgaggctcgccgttaccttgaaatgttctatgcattgaagtatcgcccattggctcaggctgttcctcttgcacaagatgattga

SEQ ID NO: 7 - DNA, 41 bp, synthetic construct
  source 1..41: mol_type = other DNA
gctaacaggaggaattaaccatggaaaataaaacggagacc

SEQ ID NO: 8 - DNA, 41 bp, synthetic construct
  source 1..41: mol_type = other DNA
ccagatctaccctcgagttacaacgatgaaatgtaagaaac

SEQ ID NO: 9 - DNA, 20 bp, synthetic construct
  source 1..20: mol_type = other DNA
ctcgagggtagatctggtac

SEQ ID NO: 10 - DNA, 20 bp, synthetic construct
  source 1..20: mol_type = other DNA
ggttaattcctcctgttagc

SEQ ID NO: 11 - DNA, 20 bp, synthetic construct
  source 1..20: mol_type = other DNA
gattatttgcacggcgtcac

SEQ ID NO: 12 - DNA, 23 bp, synthetic construct
  source 1..23: mol_type = other DNA
cttgtgggtcgttgtcgaggatg

SEQ ID NO: 13 - DNA, 41 bp, synthetic construct
  source 1..41: mol_type = other DNA
ctaacaggaggaattaaccatatggccgaaaacaagaccga

SEQ ID NO: 14 - DNA, 41 bp, synthetic construct
  source 1..41: mol_type = other DNA
gtaccagatctaccctcgagttacaaagaggaaatgtaaga

SEQ ID NO: 15 - DNA, 20 bp, synthetic construct
  source 1..20: mol_type = other DNA
ctcgagggtagatctggtac

SEQ ID NO: 16 - DNA, 20 bp, synthetic construct
  source 1..20: mol_type = other DNA
ggttaattcctcctgttagc

SEQ ID NO: 17 - DNA, 20 bp, synthetic construct
  source 1..20: mol_type = other DNA
ctgcagttccagttcacgac

SEQ ID NO: 18 - DNA, 20 bp, synthetic construct
  source 1..20: mol_type = other DNA
atggccgaaaacaagaccga

SEQ ID NO: 19 - DNA, 20 bp, synthetic construct
  source 1..20: mol_type = other DNA
ttacaaagaggaaatgtaag

SEQ ID NO: 20 - protein, 462 aa, synthetic construct
MDSGYSSSYAAAAGMHVVICPWLAFGHLLPCLDLAQRLASRGHRVSFVSTPRNISRLPPVRPALAPLVAFVALPLPRVEGLPDGAESTNDVPHDRPDMVELHRRAFDGLAAPFSEFLGTACADWVIVDVFHHWAAAAALEHKVPCAMMLLGSAHMIASIADRRLERAETESPAAAGQGRPAAAPTFEVARMKLIRTKGSSGMSLAERFSLTLSRSSLVVGRSCVEFEPETVPLLSTLRGKPITFLGLMPPLHEGRREDGEDATVRWLDAQPAKSVVYVALGSEVPLGVEKVHELALGLELAGTRFLWALRKPTGVSDADLLPAGFEERTRGRGVVATRWVPQMSILAHAAVGAFLTHCGWNSTIEGLMFGHPLIMLPIFGDQGPNARLIEAKNAGLQVARNDGDGSFDREGVAAAIRAVAVEEESSKVFQAKAKKLQEIVADMACHERYIDGFIQQLRSYKD

SEQ ID NO: 21 - DNA, 1386 bp, synthetic construct
  source 1..1386: mol_type = other DNA
atggattcgggttactcttcctcctatgcggcggctgcgggtatgcacgttgttatttgtccgtggctggcgtttggtcacctgctgccgtgcctggaccttgcacaacgtctggcttctcgtggtcaccgcgttagcttcgtctccaccccgcgtaacatttctcgtctgccgccggtacgtcctgcgttggctccgctggttgcgttcgtggcactcccgctgccgcgcgtcgagggtctgccggatggtgcggaatccaccaatgacgttccacatgatcgtccggacatggttgaactgcaccgccgtgcctttgacggtctggcagcaccgttctctgaatttctgggcaccgcttgcgctgactgggtaatcgttgatgttttccaccattgggctgctgcggcggcgctggaacacaaggtcccttgtgcaatgatgctgctgggcagcgcacacatgatcgcatccatcgcagatcgccgcctggaacgtgctgagactgaaagcccggcagcggccggtcagggtcgtccggccgcggcgccgactttcgaagtcgctcgtatgaaactgatccgcaccaaaggctcttctggtatgtcgctggctgagcgtttttccctcaccctgtcccgttccagtctggttgttggccggtcctgtgtcgagttcgaaccggaaactgttccactgctgtctacgctgcgtggtaagccgatcacttttttgggcctgatgccgccactgcacgaaggtcgtcgtgaagatggtgaagacgctactgttcgctggctggacgcgcagccagcaaaatctgtagtgtacgtagcactgggttctgaagttccgcttggcgttgagaaagtgcacgaactggcgctcggcctggaactggctggtacccgtttcctgtgggcgctgcgcaagcccactggtgtttctgacgcggatctcctgccggcgggctttgaagagcgcacacgcggtcgtggcgttgttgctactcgctgggtcccacagatgtccattctggcgcatgcggccgtgggtgcgttcctgactcattgcggctggaactctaccatcgagggtctcatgtttggccacccgctgattatgctgcctatctttggggaccagggcccgaacgcacgcctgattgaagcaaaaaacgcgggtctccaggtagctcgtaacgacggcgatggctccttcgaccgtgaaggcgtagcggcggcaatccgcgctgttgctgttgaagaagagagttctaaggtttttcaagccaaggccaaaaaattacaggagatcgtggctgacatggcatgccacgaacgttacatcgacggttttatccagcaactccgtagctataaagac

SEQ ID NO: 22 - protein, 462 aa, synthetic construct
MDSGYSSSYAAAAGMHVVICPWLAFGHLLPCLDLAQRLASRGHRVSFVSTPRNISRLPPVRPALAPLVAFVALPLPRVEGLPDGAESTYDVPHDRPDMVELHRRAFDGLAAPFSEFLGTACADWVIVDVFHHWAAAAALEHKVPCAMMLLGSAHLIASIADRRLERAETESPAAAGQGRPAAAPTFEVARMKLIRTKGSSGMSLAERFSLTLSRSSLVVGRSCVEFEPETVPLLSTLRGKPITFLGLMPPLHEGRREDGEDATVRWLDAQPAKTVVYVALGSEVPLGVEKVHELALGLELAGTRFLWALRKPTGVSDADLLPAGFEERTRGRGVVATRWVPQMSILAHAAVGAFLTHCGWSSTIEGLMFGHPLIMLPIFGDQGPNARLIEAKNAGLQVARNDGDGSFDREGVAAAIRAVAVEEESSKVFQAKAKKLQEIVADMACHERYIDGFIQQLRSYKD

SEQ ID NO: 23 - DNA, 1389 bp, synthetic construct
  source 1..1389: mol_type = other DNA
atggactccggctactcctcctcctacgccgccgccgccgggatgcacgtcgtgatctgcccgtggctcgccttcggccacctgctcccgtgcctcgacctcgcccagcgcctcgcgtcgcggggccaccgcgtgtcgttcgtctccacgccgcggaacatatcccgcctcccgccggtgcgccccgcgctcgcgccgctcgtcgccttcgtggcgctgccgctcccgcgcgtcgaggggctccccgacggcgccgagtccacctatgacgtcccccacgacaggccggacatggtcgagctccaccggagggccttcgacgggctcgccgcgcccttctcggagttcttgggcaccgcgtgcgccgactgggtcatcgtcgacgtcttccaccactgggccgcagccgccgctctcgagcacaaggtgccatgtgcaatgatgttgttgggctctgcacatttgatcgcttccatagcagacagacggctcgagcgcgcggagacagagtcgcctgcggctgccgggcagggacgcccagcggcggcgccaacgttcgaggtggcgaggatgaagttgatacgaaccaaaggctcatcgggaatgtccctcgccgagcgcttctccttgacgctctcgaggagcagcctcgtcgtcgggcggagctgcgtggagttcgagccggagaccgtcccgctcctgtcgacgctccgcggtaagcctattaccttccttggccttatgccgccgttgcatgaaggccgccgcgaggacggcgaggatgccaccgtccgctggctcgacgcgcagccggccaagacggtcgtgtacgtcgcgctaggcagcgaggtgccactgggagtggagaaggtccacgagctcgcgctcgggctggagctcgccgggacgcgcttcctctgggctcttaggaagcccactggcgtctccgacgccgacctcctccccgccggcttcgaggagcgcacgcgcggccgcggcgtcgtggcgacgagatgggttcctcagatgagcatactggcgcacgccgccgtgggcgcgttcctgacccactgcggctggagctcgaccatcgaggggctcatgttcggccacccgcttatcatgctgccgatcttcggcgaccagggaccgaacgcgcggctaatcgaggcgaagaacgccggattgcaggtggcaagaaacgacggcgatggatcgttcgaccgagaaggcgtcgcggcggcgattcgtgcagtcgcggtggaggaagaaagcagcaaagtgtttcaagccaaagccaagaagctgcaggagatcgtcgcggacatggcctgccatgagaggtacatcgacggattcattcagcaattgagatcttacaaggattga

SEQ ID NO: 24 - DNA, 41 bp, synthetic construct
  source 1..41: mol_type = other DNA
ctttaagaaggagatataccatggattcgggttactcttcc

SEQ ID NO: 25 - DNA, 43 bp, synthetic construct
  source 1..43: mol_type = other DNA
cttgtcgacggagctcgaattcttagtctttatagctacggag

SEQ ID NO: 26 - DNA, 22 bp, synthetic construct
  source 1..22: mol_type = other DNA
gaattcgagctccgtcgacaag

SEQ ID NO: 27 - DNA, 20 bp, synthetic construct
  source 1..20: mol_type = other DNA
ggtatatctccttcttaaag

SEQ ID NO: 28 - DNA, 20 bp, synthetic construct
  source 1..20: mol_type = other DNA
taatacgactcactataggg

SEQ ID NO: 29 - DNA, 20 bp, synthetic construct
  source 1..20: mol_type = other DNA
ggcggtgcagttcaaccatg

SEQ ID NO: 30 - protein, 459 aa, synthetic construct
MAENKTETTVRRRRRIILFPVPFQGHINPILQLANVLYSKGFSITIFHTNFNKPKTSNYPHFTFRFILDNDPQDERISNLPTHGPLAGHRIPIINEHGADELRRELELLMLASEEDEEVSCLITDALWYFAQSVADSLNLRRLVLMTSSLFNFHAHVSLPQFDELGYLDPDDKTRLEEQASGFPMLKVKDIKSAYSNWQILKEILGKMIKQTKASSGVIWNSFKELEESELETVIREIPAPSFLIPLPKHLTASSSSLLDHDRTVFQWLDQQPPSSVLYVSFGSTSEVDEKDFLEIARGLVDSKQSFLWVVRPGFVKGSTWVEPLPDGFLGERGRIVKWVPQQEVLAHGAIGAFWTHSGWNSTLESVCEGVPMIFSDFGMDQPLNARYMSDVLKVGVYLENGWERGEIANYIRRVMVDEEGEYIRQNARVLKQKADVSLMKGGSSYESLESLVSYISSL

SEQ ID NO: 31 - DNA, 1380 bp, synthetic construct
  source 1..1380: mol_type = other DNA
atggccgaaaataaaacggagaccaccgttcgccggcgccggagaataatattattcccggtaccatttcaaggccacattaacccaattcttcagctagccaatgtgttgtactctaaaggattcagtatcaccatctttcacaccaacttcaacaaacccaaaacatctaattaccctcacttcactttcagattcatcctcgacaacgacccacaagacgaacgcatttccaatctaccgactcatggtccgctcgctggtcatcggattccgattatcaacgaacacggagctgacgaattacgacgcgaactggaactgctgatgttagctagcgaagaagatgaagaggtatcgtgtttaatcacggatgctctttggtacttcgcgcaatctgttgctgacagtcttaacctccgacggcttgttttgatgacaagcagcttgtttaattttcatgcacatgtttcacttcctcagtttgatgagcttggttacctcgatcctgatgacaaaacccgtttggaagaacaagcgagtgggtttcctatgctaaaagtgaaagacatcaagtctgcgtatagcaactggcaaatactcaaagagatattagggaagatgataaaacaaacaaaagcatcttcaggagtcatctggaactcatttaaggaactcgaagagtctgagctcgaaactgttatccgtgagatcccggctccaagtttcttgataccactccccaagcatttgacagcctcttccagcagcttactagaccacgatcgaaccgtttttcaatggttagaccaacaaccgccaagttcggtactgtatgttagttttggtagtactagtgaagtggatgagaaagatttcttggaaatagctcgtgggttggttgatagcaagcagtcgtttttatgggtggttcgacctgggtttgtcaagggttcgacgtgggtcgaaccgttgccagatgggttcttgggtgaaagaggacgtattgtgaaatgggttccacagcaagaagtgctagctcatggagcaataggcgcattctggactcatagcggatggaactctacgttggaaagcgtttgtgaaggtgttcctatgattttctcggattttgggatggatcaaccgttgaatgctagatacatgagtgatgttttgaaggtaggggtgtatttggaaaatgggtgggaaagaggagagatagcaaattatataagaagagttatggtggatgaagaaggagaatacatcagacagaatgcaagagttttgaaacaaaaggcagatgtttctttgatgaagggtggttcgtcttacgaatcattagagtctctagtttcttacatttcatcgttgtaa

SEQ ID NO: 32 - DNA, 40 bp, synthetic construct
  source 1..40: mol_type = other DNA
gtaccagatctaccctcgagttacaaagaggaaatgtaag